European Patent Specification EP 3 921 422 B1, published November 22, 2023. Title: Chloride-inducible prokaryotic expression system. Applicant: Aurealis Pharma AG. The sequence listing filed with the application follows.

SEQUENCE LISTING (36 sequences)

SEQ ID NO: 1 - DNA, 3201 bp, Artificial Sequence
  plasmid pAUC1010
agatctcatgacggagtttattcttgacacaggtatggacttatgatataataaaacagtactctgcaggcatgcggtaccactagttctagagagctcaagctttctttgaaccaaaattagaaaaccaaggcttgaaacgttcaattgaaatggcaattaaacaaattacagcacgtgttgctttgattgatagccaaaaagcagcagttgataaagcaattactgatattgctgaaaaattgtaatttataaataaaaatcaccttttagaggtggtttttttatttataaattattcgtttgatttcgctttcgatagaacaatcaaatcgtttctgagacgttttagcgtttatttcgtttagttatcggcataatcgttaaaacaggcgttatcgtagcgtaaaagcccttgagcgtagcgtggctttgcagcgaagatgttgtctgttagattatgaaagccgatgactgaatgaaataataagcgcagcgtccttctatttcggttggaggaggctcaagggagtttgagggaatgaaattccctcatgggtttgattttaaaaattgcttgcaattttgccgagcggtagcgctggaaaatttttgaaaaaaatttggaatttggaaaaaaatggggggaaaggaagcgaattttgcttccgtactacgaccccccattaagtgccgagtgccaatttttgtgccaaaaacgctctatcccaactggctcaagggtttgaggggtttttcaatcgccaacgaatcgccaacgttttcgccaacgttttttataaatctatatttaagtagctttatttttgtttttatgattacaaagtgatacactaattttataaaattatttgattggagttttttaaatggtgatttcagaatcgaaaaaaagagttatgatttctctgacaaaagagcaagataaaaaattaacagatatggcgaaacaaaaagatttttcaaaatctgcggttgcggcgttagctatagaagaatatgcaagaaaggaatcagaacaaaaaaaataagcgaaagctcgcgtttttagaaggatacgagttttcgctacttgtttttgataaggtaattatatcatggctattaaaaatactaaagctagaaattttggatttttattatatcctgactcaattcctaatgattggaaagaaaaattagagagtttgggcgtatctatggctgtcagtcctttacacgatatggacgaaaaaaaagataaagatacatggaatagtagtgatgttatacgaaatggaaagcactataaaaaaccacactatcacgttatatatattgcacgaaatcctgtaacaatagaaagcgttaggaacaagattaagcgaaaattggggaatagttcagttgctcatgttgagatacttgattatatcaaaggttcatatgaatatttgactcatgaatcaaaggacgctattgctaagaataaacatatatacgacaaaaaagatattttgaacattaatgattttgatattgaccgctatataacacttgatgaaagccaaaaaagagaattgaagaatttacttttagatatagtggatgactataatttggtaaatacaaaagatttaatggcttttattcgccttaggggagcggagtttggaattttaaatacgaatgatgtaaaagatattgtttcaacaaactctagcgcctttagattatggtttgagggcaattatcagtgtggatatagagcaagttatgcaaaggttcttgatgctgaaacgggggaaataaaatgacaaacaaagaaaaagagttatttgctgaaaatgaggaattaaaaaaagaaattaaggacttaaaagagcgtattgaaagatacagagaaatggaagttgaattaagtacaacaatagatttattgagaggagggattattgaataaataaaagcccccctgacgaaagtcgacatggtcgatgtctagatgcttaaactagagaaaggtttaaaagatgaaaacttcaccacatcgtaatacttcagctattgttgatttaaaagcgattagaaataatattgaaaaatttaaaaagcatattaaccctaatgcagagatttggccagcagtgaaagcagatgcttatggtcatggctcgattgaggtttctaaagcggtgagcgatttggtaggtggtttttgtgtatcaaacctagatgaggcaattgaattacgaaatcatctggtgactaaaccgattttagttttatccggaattgttccagaagatgttgatattgcagctgcccttaatattagtcttactgccccgagtttagaatggttgaaattggttgttcaagaagaagcagaactttcagatttaaaaattcatattggtgtagattctggtatgggtcggattggtattcgtgatgttgaagaagctaatcagatgattgaacttgctgataaatatgcgattaattttgaaggaattttcactcattttgcgactgcggatatggctgatgaaacaaaatttaaaaatcaacaggcaagatttaacaaaattatggccggattatcacgtcaaccaaaatttatacactcaactaatacggccgctgctttatggcataaggaacaagttcaagctattgaacgtttagggatttcaatgtatggcttgaatccaagtggtaaaactttggaacttccttttgaaattgaacccgctctctctttagtttctgaattgactcatataaaaaaaatagctgcaggtgaaacggttggttatggtgcaacttatgagacgagtgaagaaacttggattggaactgttccaattggttacgctgacgggtggacccgtcaaatgcaaggtttcaaagtgcttgttgatggaaagttttgtgagattgttggtcgagtttgtatggatcaaatgatgataaaacttgataagtcttaccctttgggaacgaaggtcactttgattggtcgagataaggctaatgaaatcacgacaacagacgttgctgattggcgtggaacgattaattatgaagtgctttgcttactttctgatagaatcaaaagaatctataaataaaattaaaaaaactgtatttttacagtttttttgttttctgttaaaagcagatgataacctcact

SEQ ID NO: 2 - DNA, 1248 bp, Lactococcus lactis
  PgadC promoter
tgagcgttgtataagcttttatgtctttctatatcaacttttaatagaaatataaagtaatataaatgtttttataataaattatgtgagatatatttttttgtccgtactggtatagatttgacgattaagtcttaaataagttataatctcaattgcgtaatttcttaaatacagaaataacaactacattggtagactgattaaaaagtgtacttgatgaactgttataaaccttaaaaaaataaaaataatagtttgggggatgttaaagatgtataaaaaatatggagattgttttaaaaagttgcgaaaccaaaagaatttagggttatcatactttagtaaacttggaatagaccgttcaaatatatctagatttgaacatggaaaatgtatgatgagttttgagcgtatagatttgatgttagaagaaatgcaagttccgttatctgagtacgaattgattgtaaataattttatgccgaatttccaagaattttttatattagaattggaaaaagctgaatttagccaaaatcgagataaaataaaagagttgtattctgaggtcaaagaaacggggaatcatttactgacggttaccgtgaaaacgaagcttgggaatataagtcagacagaagttaaagaaattgaagcttatctttgcaatattgaagagtggggatattttgaacttactttattttattttgtatctgattatctcaatgtcaatcaattagaattgctgctttttaattttgataaaagatgtgaaaattactgtagagtcttaaaatatagaaggagactattgcaaatagcctataaaagtgttgcgatatacgcggctaaaggagaaagaaaaaaagccgaaaatattttagaaatgactaaaaaatatcgaactgtgggagtcgatttatattcagaagtattaagacatcttgctagagctatcattatttttaattttgaaaatgcagagattggggaagaaaaaataaattatgctcttgagattttggaagaatttggaggaaagaagataaaagaattctatcagaataaaatggaaaagtatttgaaaaggtcaatttagtctcttttgagctgttgctttaaagcaacagctcaaaagagattttctttattctagagcatatactagagggtgaagataggttgtctgaagcattataacttgtcttttaaaaaattcaatcataaatataaggaggtatg

SEQ ID NO: 3 - protein, 27 aa, Lactococcus lactis
  Usp45 secretion signal
MKKKIISAILMSTVILSAAAPLSGVYA

SEQ ID NO: 4 - RNA, 16 nt, Lactococcus lactis
  3’ end of 16S RNA
ggaucaccuccuuucu

SEQ ID NO: 5 - protein, 155 aa, Homo sapiens [sequence omitted]

SEQ ID NO: 6 - protein, 153 aa, Artificial Sequence
  recombinant hFGF-2 variant
AGSITTLPALPEDGGSGAFPPGHFKDPKRLYCKNGGFFLRIHPDGRVDGVREKSDPHIKLQLQAEERGVVSIKGVCANRYLAMKEDGRLLASKCVTDECFFFERLESNNYNTYRSRKYTSWYVALKRTGQYKLGSKTGPGQKAILFLPMSAKS

SEQ ID NO: 7 - protein, 180 aa, Artificial Sequence
  recombinant hFGF-2-153 precursor protein
MKKKIISAILMSTVILSAAAPLSGVYAAGSITTLPALPEDGGSGAFPPGHFKDPKRLYCKNGGFFLRIHPDGRVDGVREKSDPHIKLQLQAEERGVVSIKGVCANRYLAMKEDGRLLASKCVTDECFFFERLESNNYNTYRSRKYTSWYVALKRTGQYKLGSKTGPGQKAILFLPMSAKS

SEQ ID NO: 8 - protein, 129 aa, Homo sapiens [sequence omitted]

SEQ ID NO: 9 - protein, 130 aa, Artificial Sequence
  recombinant hIL-4 variant
AHKCDITLQEIIKTLNSLTEQKTLCTELTVTDIFAASKNTTEKETFCRAATVLRQFYSHHEKDTRCLGATAQQFHRHKQLIRFLKRLDRNLWGLAGLNSCPVKEANQSTLENFLERLKTIMREKYSKCSS

SEQ ID NO: 10 - protein, 157 aa, Artificial Sequence
  recombinant hIL-4 precursor protein
MKKKIISAILMSTVILSAAAPLSGVYAAHKCDITLQEIIKTLNSLTEQKTLCTELTVTDIFAASKNTTEKETFCRAATVLRQFYSHHEKDTRCLGATAQQFHRHKQLIRFLKRLDRNLWGLAGLNSCPVKEANQSTLENFLERLKTIMREKYSKCSS

SEQ ID NO: 11 - protein, 418 aa, Homo sapiens
  mature form of human colony stimmulating factor 1 (CSF-1)
EEVSEYCSHMIGSGHLQSLQRLIDSQMETSCQITFEFVDQEQLKDPVCYLKKAFLLVQDIMEDTMRFRDNTPNAIAIVQLQELSLRLKSCFTKDYEEHDKACVRTFYETPLQLLEKVKNVFNETKNLLDKDWNIFSKNCNNSFAECSSQDVVTKPDCNCLYPKAIPSSDPASVSPHQPLAPSMAPVAGLTWEDSEGTEGSSLLPGEQPLHTVDPGSAKQRPPRSTCQSFEPPETPVVKDSTIGGSPQPRPSVGAFNPGMEDILDSAMGTNWVPEEASGEASEIPVPQGTELSPSRPGGGSMQTEPARPSNFLSASSPLPASAKGQQPADVTGTALPRVGPVRPTGQDWNHTPQKTDHPSALLRDPPEPGSPRISSLRPQGLSNPSTLSAQPQLSRSHSSGSVLPLGELEGRRSTRDRR

SEQ ID NO: 12 - protein, 159 aa, Artificial Sequence
  recombinant hCSF-1 variant
AEEVSEYCSHMIGSGHLQSLQRLIDSQMETSCQITFEFVDQEQLKDPVCYLKKAFLLVQDIMEDTMRFRDNTPNAIAIVQLQELSLRLKSCFTKDYEEHDKACVRTFYETPLQLLEKVKNVFNETKNLLDKDWNIFSKNCNNSFAECSSQGHERQSEGS

SEQ ID NO: 13 - protein, 186 aa, Artificial Sequence
  recombinant hCSF-1 precursor protein
MKKKIISAILMSTVILSAAAPLSGVYAAEEVSEYCSHMIGSGHLQSLQRLIDSQMETSCQITFEFVDQEQLKDPVCYLKKAFLLVQDIMEDTMRFRDNTPNAIAIVQLQELSLRLKSCFTKDYEEHDKACVRTFYETPLQLLEKVKNVFNETKNLLDKDWNIFSKNCNNSFAECSSQGHERQSEGS

SEQ ID NO: 14 - DNA, 2899 bp, Artificial Sequence
  synthetic CFI construct
agatctgagcgttgtataagcttttatgtctttctatatcaacttttaatagaaatataaagtaatataaatgtttttataataaattatgtgagatatatttttttgtccgtactggtatagatttgacgattaagtcttaaataagttataatctcaattgcgtaatttcttaaatacagaaataacaactacattggtagactgattaaaaagtgtacttgatgaactgttataaaccttaaaaaaataaaaataatagtttgggggatgttaaagatgtataaaaaatatggagattgttttaaaaagttgcgaaaccaaaagaatttagggttatcatactttagtaaacttggaatagaccgttcaaatatatctagatttgaacatggaaaatgtatgatgagttttgagcgtatagatttgatgttagaagaaatgcaagttccgttatctgagtacgaattgattgtaaataattttatgccgaatttccaagaattttttatattagaattggaaaaagctgaatttagccaaaatcgagataaaataaaagagttgtattctgaggtcaaagaaacggggaatcatttactgacggttaccgtgaaaacgaagcttgggaatataagtcagacagaagttaaagaaattgaagcttatctttgcaatattgaagagtggggatattttgaacttactttattttattttgtatctgattatctcaatgtcaatcaattagaattgctgctttttaattttgataaaagatgtgaaaattactgtagagtcttaaaatatagaaggagactattgcaaatagcctataaaagtgttgcgatatacgcggctaaaggagaaagaaaaaaagccgaaaatattttagaaatgactaaaaaatatcgaactgtgggagtcgatttatattcagaagtattaagacatcttgctagagctatcattatttttaattttgaaaatgcagagattggggaagaaaaaataaattatgctcttgagattttggaagaatttggaggaaagaagataaaagaattctatcagaataaaatggaaaagtatttgaaaaggtcaatttagtctcttttgagctgttgctttaaagcaacagctcaaaagagattttctttattctagagcatatactagagggtgaagataggttgtctgaagcattataacttgtcttttaaaaaattcaatcataaatataaggaggtatgatgaaaaagaaaatcatttcagcgattttgatgtcaacggttattttaagcgcagcagctccattatctggagtttatgcagcagaagaagttagtgagtactgtagtcatatgattggttctggacacttacaatcacttcagcgtcttattgatagtcaaatggaaacctcttgtcaaattacatttgaatttgtagaccaagaacaacttaaagatccagtatgttatcttaagaaagcttttcttttagtccaagacataatggaagatacaatgagattcagagacaatactcctaacgctatcgccattgtccaattacaagaactttctttaagattgaaaagttgcttcactaaagattatgaggaacatgataaagcttgtgttcgaacattttatgaaactcctttgcaattattggaaaaagtgaaaaatgttttcaatgagacgaagaatttgttggataaagattggaatatattcagtaagaattgtaataactcatttgccgaatgttcaagccagggtcatgaacgtcaatcagaaggctcttaataaacgcgtattaataaggaggctaactaatgaaaaaaaagattatctcagctattttaatgtctacagtgatactttctgctgcagccccgttgtcaggtgtttacgctgctggttccattacgaccttgccggctttaccagaggacggaggttcaggagcctttccaccagggcactttaaagatcccaaacgtctatattgtaaaaatggaggcttctttctgcgaattcatcctgatggacgtgtagatggtgtgcgtgagaaaagtgatcctcatatcaaactccaacttcaggcagaagaaagaggcgtcgtaagtataaaaggagtttgcgcgaatcgttacttagctatgaaagaagacggtcgattattggcctctaagtgtgttactgatgaatgttttttttttgaacggcttgaatctaataattataacacttatagaagcagaaaatatacatcatggtacgttgcacttaaaaggacaggtcaatataaattagggtctaagacaggacctggtcaaaaagcaattttgttcttaccaatgtcggctaaaagttaataaacgcgtgaaatttaggaggtagtccaaatgaagaaaaagattattagtgcaattttaatgtcaacggtcatcttaagcgctgctgccccattgtcaggtgtttatgcagcacataagtgtgatataacattacaagaaattatcaaaacccttaatagtttaactgaacagaagactttgtgtaccgaattaactgtaactgatatttttgctgcttctaaaaatacaactgaaaaagagacattttgtcgagctgccacagtgttaagacaattttacagtcatcatgaaaaagacacaagatgtcttggtgctacggcacaacaatttcatagacacaaacaacttatccgttttcttaaacgtttggatcgtaatctgtggggcttggcaggattgaacagttgtcctgttaaagaagccaatcaatctactcttgaaaatttcttagagagattgaaaacaattatgcgagaaaaatattctaagtgttcatcttaataagcatgc

SEQ ID NO: 15 - DNA, 6025 bp, Artificial Sequence
  plasmid pC-CFI
agatctgagcgttgtataagcttttatgtctttctatatcaacttttaatagaaatataaagtaatataaatgtttttataataaattatgtgagatatatttttttgtccgtactggtatagatttgacgattaagtcttaaataagttataatctcaattgcgtaatttcttaaatacagaaataacaactacattggtagactgattaaaaagtgtacttgatgaactgttataaaccttaaaaaaataaaaataatagtttgggggatgttaaagatgtataaaaaatatggagattgttttaaaaagttgcgaaaccaaaagaatttagggttatcatactttagtaaacttggaatagaccgttcaaatatatctagatttgaacatggaaaatgtatgatgagttttgagcgtatagatttgatgttagaagaaatgcaagttccgttatctgagtacgaattgattgtaaataattttatgccgaatttccaagaattttttatattagaattggaaaaagctgaatttagccaaaatcgagataaaataaaagagttgtattctgaggtcaaagaaacggggaatcatttactgacggttaccgtgaaaacgaagcttgggaatataagtcagacagaagttaaagaaattgaagcttatctttgcaatattgaagagtggggatattttgaacttactttattttattttgtatctgattatctcaatgtcaatcaattagaattgctgctttttaattttgataaaagatgtgaaaattactgtagagtcttaaaatatagaaggagactattgcaaatagcctataaaagtgttgcgatatacgcggctaaaggagaaagaaaaaaagccgaaaatattttagaaatgactaaaaaatatcgaactgtgggagtcgatttatattcagaagtattaagacatcttgctagagctatcattatttttaattttgaaaatgcagagattggggaagaaaaaataaattatgctcttgagattttggaagaatttggaggaaagaagataaaagaattctatcagaataaaatggaaaagtatttgaaaaggtcaatttagtctcttttgagctgttgctttaaagcaacagctcaaaagagattttctttattctagagcatatactagagggtgaagataggttgtctgaagcattataacttgtcttttaaaaaattcaatcataaatataaggaggtatgatgaaaaagaaaatcatttcagcgattttgatgtcaacggttattttaagcgcagcagctccattatctggagtttatgcagcagaagaagttagtgagtactgtagtcatatgattggttctggacacttacaatcacttcagcgtcttattgatagtcaaatggaaacctcttgtcaaattacatttgaatttgtagaccaagaacaacttaaagatccagtatgttatcttaagaaagcttttcttttagtccaagacataatggaagatacaatgagattcagagacaatactcctaacgctatcgccattgtccaattacaagaactttctttaagattgaaaagttgcttcactaaagattatgaggaacatgataaagcttgtgttcgaacattttatgaaactcctttgcaattattggaaaaagtgaaaaatgttttcaatgagacgaagaatttgttggataaagattggaatatattcagtaagaattgtaataactcatttgccgaatgttcaagccagggtcatgaacgtcaatcagaaggctcttaataaacgcgtattaataaggaggctaactaatgaaaaaaaagattatctcagctattttaatgtctacagtgatactttctgctgcagccccgttgtcaggtgtttacgctgctggttccattacgaccttgccggctttaccagaggacggaggttcaggagcctttccaccagggcactttaaagatcccaaacgtctatattgtaaaaatggaggcttctttctgcgaattcatcctgatggacgtgtagatggtgtgcgtgagaaaagtgatcctcatatcaaactccaacttcaggcagaagaaagaggcgtcgtaagtataaaaggagtttgcgcgaatcgttacttagctatgaaagaagacggtcgattattggcctctaagtgtgttactgatgaatgttttttttttgaacggcttgaatctaataattataacacttatagaagcagaaaatatacatcatggtacgttgcacttaaaaggacaggtcaatataaattagggtctaagacaggacctggtcaaaaagcaattttgttcttaccaatgtcggctaaaagttaataaacgcgtgaaatttaggaggtagtccaaatgaagaaaaagattattagtgcaattttaatgtcaacggtcatcttaagcgctgctgccccattgtcaggtgtttatgcagcacataagtgtgatataacattacaagaaattatcaaaacccttaatagtttaactgaacagaagactttgtgtaccgaattaactgtaactgatatttttgctgcttctaaaaatacaactgaaaaagagacattttgtcgagctgccacagtgttaagacaattttacagtcatcatgaaaaagacacaagatgtcttggtgctacggcacaacaatttcatagacacaaacaacttatccgttttcttaaacgtttggatcgtaatctgtggggcttggcaggattgaacagttgtcctgttaaagaagccaatcaatctactcttgaaaatttcttagagagattgaaaacaattatgcgagaaaaatattctaagtgttcatcttaataagcatgcggtaccactagttctagagagctcaagctttctttgaaccaaaattagaaaaccaaggcttgaaacgttcaattgaaatggcaattaaacaaattacagcacgtgttgctttgattgatagccaaaaagcagcagttgataaagcaattactgatattgctgaaaaattgtaatttataaataaaaatcaccttttagaggtggtttttttatttataaattattcgtttgatttcgctttcgatagaacaatcaaatcgtttctgagacgttttagcgtttatttcgtttagttatcggcataatcgttaaaacaggcgttatcgtagcgtaaaagcccttgagcgtagcgtggctttgcagcgaagatgttgtctgttagattatgaaagccgatgactgaatgaaataataagcgcagcgtccttctatttcggttggaggaggctcaagggagtttgagggaatgaaattccctcatgggtttgattttaaaaattgcttgcaattttgccgagcggtagcgctggaaaatttttgaaaaaaatttggaatttggaaaaaaatggggggaaaggaagcgaattttgcttccgtactacgaccccccattaagtgccgagtgccaatttttgtgccaaaaacgctctatcccaactggctcaagggtttgaggggtttttcaatcgccaacgaatcgccaacgttttcgccaacgttttttataaatctatatttaagtagctttatttttgtttttatgattacaaagtgatacactaattttataaaattatttgattggagttttttaaatggtgatttcagaatcgaaaaaaagagttatgatttctctgacaaaagagcaagataaaaaattaacagatatggcgaaacaaaaagatttttcaaaatctgcggttgcggcgttagctatagaagaatatgcaagaaaggaatcagaacaaaaaaaataagcgaaagctcgcgtttttagaaggatacgagttttcgctacttgtttttgataaggtaattatatcatggctattaaaaatactaaagctagaaattttggatttttattatatcctgactcaattcctaatgattggaaagaaaaattagagagtttgggcgtatctatggctgtcagtcctttacacgatatggacgaaaaaaaagataaagatacatggaatagtagtgatgttatacgaaatggaaagcactataaaaaaccacactatcacgttatatatattgcacgaaatcctgtaacaatagaaagcgttaggaacaagattaagcgaaaattggggaatagttcagttgctcatgttgagatacttgattatatcaaaggttcatatgaatatttgactcatgaatcaaaggacgctattgctaagaataaacatatatacgacaaaaaagatattttgaacattaatgattttgatattgaccgctatataacacttgatgaaagccaaaaaagagaattgaagaatttacttttagatatagtggatgactataatttggtaaatacaaaagatttaatggcttttattcgccttaggggagcggagtttggaattttaaatacgaatgatgtaaaagatattgtttcaacaaactctagcgcctttagattatggtttgagggcaattatcagtgtggatatagagcaagttatgcaaaggttcttgatgctgaaacgggggaaataaaatgacaaacaaagaaaaagagttatttgctgaaaatgaggaattaaaaaaagaaattaaggacttaaaagagcgtattgaaagatacagagaaatggaagttgaattaagtacaacaatagatttattgagaggagggattattgaataaataaaagcccccctgacgaaagtcgacatggtcgatgtctagatgcttaaactagagaaaggtttaaaagatgaaaacttcaccacatcgtaatacttcagctattgttgatttaaaagcgattagaaataatattgaaaaatttaaaaagcatattaaccctaatgcagagatttggccagcagtgaaagcagatgcttatggtcatggctcgattgaggtttctaaagcggtgagcgatttggtaggtggtttttgtgtatcaaacctagatgaggcaattgaattacgaaatcatctggtgactaaaccgattttagttttatccggaattgttccagaagatgttgatattgcagctgcccttaatattagtcttactgccccgagtttagaatggttgaaattggttgttcaagaagaagcagaactttcagatttaaaaattcatattggtgtagattctggtatgggtcggattggtattcgtgatgttgaagaagctaatcagatgattgaacttgctgataaatatgcgattaattttgaaggaattttcactcattttgcgactgcggatatggctgatgaaacaaaatttaaaaatcaacaggcaagatttaacaaaattatggccggattatcacgtcaaccaaaatttatacactcaactaatacggccgctgctttatggcataaggaacaagttcaagctattgaacgtttagggatttcaatgtatggcttgaatccaagtggtaaaactttggaacttccttttgaaattgaacccgctctctctttagtttctgaattgactcatataaaaaaaatagctgcaggtgaaacggttggttatggtgcaacttatgagacgagtgaagaaacttggattggaactgttccaattggttacgctgacgggtggacccgtcaaatgcaaggtttcaaagtgcttgttgatggaaagttttgtgagattgttggtcgagtttgtatggatcaaatgatgataaaacttgataagtcttaccctttgggaacgaaggtcactttgattggtcgagataaggctaatgaaatcacgacaacagacgttgctgattggcgtggaacgattaattatgaagtgctttgcttactttctgatagaatcaaaagaatctataaataaaattaaaaaaactgtatttttacagtttttttgttttctgttaaaagcagatgataacctcact

SEQ ID NO: 16 - protein, 157 aa, Mus musculus
  mature form of mouse interleukin 18 (mIL-18)
NFGRLHCTTAVIRNINDQVLFVDKRQPVFEDMTDIDQSASEPQTRLIIYMYKDSEVRGLAVTLSVKDSKMSTLSCKNKIISFEEMDPPENIDDIQSDLIFFQKRVPGHNKMEFESSLYEGHFLACQKEDDAFKLILKKKDENGDKSVMFTLTNLHQS

SEQ ID NO: 17 - protein, 158 aa, Artificial Sequence
  recombinant variant of mIL-18
ANFGRLHCTTAVIRNINDQVLFVDKRQPVFEDMTDIDQSASEPQTRLIIYMYKDSEVRGLAVTLSVKDSKMSTLSCKNKIISFEEMDPPENIDDIQSDLIFFQKRVPGHNKMEFESSLYEGHFLACQKEDDAFKLILKKKDENGDKSVMFTLTNLHQS

SEQ ID NO: 18 - protein, 185 aa, Artificial Sequence
  recombinant mIL-18 precusor protein
MKKKIISAILMSTVILSAAAPLSGVYAANFGRLHCTTAVIRNINDQVLFVDKRQPVFEDMTDIDQSASEPQTRLIIYMYKDSEVRGLAVTLSVKDSKMSTLSCKNKIISFEEMDPPENIDDIQSDLIFFQKRVPGHNKMEFESSLYEGHFLACQKEDDAFKLILKKKDENGDKSVMFTLTNLHQS

SEQ ID NO: 19 - protein, 125 aa, Mus musculus
  mature form of mouse granulocyte-macrophage colony-stimulating factor (GM-CSF)
SAPTRSPITVTRPWKHVEAIKEALNLLDDMPVTLNEEVEVVSNEFSFKKLTCVQTRLKIFEQGLRGNFTKLKGALNMTASYYQTYCPPTPETDCETQVTTYADFIDSLKTFLTDIPFECKKPGQK

SEQ ID NO: 20 - protein, 125 aa, Artificial Sequence
  recombinant variant of mGM-CSF
AAPTRSPITVTRPWKHVEAIKEALNLLDDMPVTLNEEVEVVSNEFSFKKLTCVQTRLKIFEQGLRGNFTKLKGALNMTASYYQTYCPPTPETDCETQVTTYADFIDSLKTFLTDIPFECKKPGQK

SEQ ID NO: 21 - protein, 152 aa, Artificial Sequence
  recombinant mGM-CSF precursor protein
MKKKIISAILMSTVILSAAAPLSGVYAAAPTRSPITVTRPWKHVEAIKEALNLLDDMPVTLNEEVEVVSNEFSFKKLTCVQTRLKIFEQGLRGNFTKLKGALNMTASYYQTYCPPTPETDCETQVTTYADFIDSLKTFLTDIPFECKKPGQK

SEQ ID NO: 22 - DNA, 2309 bp, Artificial Sequence
  synthetic mEG construct
agatctgagcgttgtataagcttttatgtctttctatatcaacttttaatagaaatataaagtaatataaatgtttttataataaattatgtgagatatatttttttgtccgtactggtatagatttgacgattaagtcttaaataagttataatctcaattgcgtaatttcttaaatacagaaataacaactacattggtagactgattaaaaagtgtacttgatgaactgttataaaccttaaaaaaataaaaataatagtttgggggatgttaaagatgtataaaaaatatggagattgttttaaaaagttgcgaaaccaaaagaatttagggttatcatactttagtaaacttggaatagaccgttcaaatatatctagatttgaacatggaaaatgtatgatgagttttgagcgtatagatttgatgttagaagaaatgcaagttccgttatctgagtacgaattgattgtaaataattttatgccgaatttccaagaattttttatattagaattggaaaaagctgaatttagccaaaatcgagataaaataaaagagttgtattctgaggtcaaagaaacggggaatcatttactgacggttaccgtgaaaacgaagcttgggaatataagtcagacagaagttaaagaaattgaagcttatctttgcaatattgaagagtggggatattttgaacttactttattttattttgtatctgattatctcaatgtcaatcaattagaattgctgctttttaattttgataaaagatgtgaaaattactgtagagtcttaaaatatagaaggagactattgcaaatagcctataaaagtgttgcgatatacgcggctaaaggagaaagaaaaaaagccgaaaatattttagaaatgactaaaaaatatcgaactgtgggagtcgatttatattcagaagtattaagacatcttgctagagctatcattatttttaattttgaaaatgcagagattggggaagaaaaaataaattatgctcttgagattttggaagaatttggaggaaagaagataaaagaattctatcagaataaaatggaaaagtatttgaaaaggtcaatttagtctcttttgagctgttgctttaaagcaacagctcaaaagagattttctttattctagagcatatactagagggtgaagataggttgtctgaagcattataacttgtcttttaaaaaattcaatcataaatataaggaggtatgatgaagaaaaagattattagtgcaattttaatgtcaacggtcatcttaagcgctgctgccccattgtcaggtgtttatgcagcaaattttggtagattacattgtacaacagcagtaatacgtaatattaatgatcaagttttatttgttgataaaagacaacctgtttttgaagatatgactgatattgatcaatctgcatctgaaccacaaactagattaataatttatatgtataaagatagtgaagttagaggattagctgtaacattaagtgttaaagatagtaaaatgagtacattatcatgtaaaaacaaaataatttcatttgaagaaatggacccacctgaaaatattgatgatattcaatcagatttaattttctttcaaaaacgtgttccaggtcataacaaaatggaatttgaatctagtttatatgaaggtcactttttagcttgtcaaaaagaagatgatgcttttaaattaattttaaagaaaaaagatgaaaatggagataaatcagttatgtttacattaactaatttacatcaatcataataaacgcgtattaataaggaggctaactaatgaaaaagaaaatcatttcagcgattttgatgtcaacggttattttaagcgcagcagctccattatctggagtttatgcagccccaacacgtagtccaataacagtaactagaccttggaaacatgttgaagcaattaaagaagcattaaatttattagatgatatgccagtaacattaaatgaagaagttgaagtagtaagtaatgaatttagttttaaaaaattaacatgtgttcaaactagattaaaaatttttgaacaaggattaagaggtaattttactaaattaaaaggtgctttaaatatgacagctagttattatcaaacatattgtccaccaacacctgaaactgattgtgaaacacaagtaactacatatgctgattttattgattcattaaaaacatttttaactgatattccttttgaatgtaaaaaaccaggacaaaaataataataaggcatgc

SEQ ID NO: 23 - DNA, 5432 bp, Artificial Sequence
  plasmid pC-mEG
gatctgagcgttgtataagcttttatgtctttctatatcaacttttaatagaaatataaagtaatataaatgtttttataataaattatgtgagatatatttttttgtccgtactggtatagatttgacgattaagtcttaaataagttataatctcaattgcgtaatttcttaaatacagaaataacaactacattggtagactgattaaaaagtgtacttgatgaactgttataaaccttaaaaaaataaaaataatagtttgggggatgttaaagatgtataaaaaatatggagattgttttaaaaagttgcgaaaccaaaagaatttagggttatcatactttagtaaacttggaatagaccgttcaaatatatctagatttgaacatggaaaatgtatgatgagttttgagcgtatagatttgatgttagaagaaatgcaagttccgttatctgagtacgaattgattgtaaataattttatgccgaatttccaagaattttttatattagaattggaaaaagctgaatttagccaaaatcgagataaaataaaagagttgtattctgaggtcaaagaaacggggaatcatttactgacggttaccgtgaaaacgaagcttgggaatataagtcagacagaagttaaagaaattgaagcttatctttgcaatattgaagagtggggatattttgaacttactttattttattttgtatctgattatctcaatgtcaatcaattagaattgctgctttttaattttgataaaagatgtgaaaattactgtagagtcttaaaatatagaaggagactattgcaaatagcctataaaagtgttgcgatatacgcggctaaaggagaaagaaaaaaagccgaaaatattttagaaatgactaaaaaatatcgaactgtgggagtcgatttatattcagaagtattaagacatcttgctagagctatcattatttttaattttgaaaatgcagagattggggaagaaaaaataaattatgctcttgagattttggaagaatttggaggaaagaagataaaagaattctatcagaataaaatggaaaagtatttgaaaaggtcaatttagtctcttttgagctgttgctttaaagcaacagctcaaaagagattttctttattctagagcatatactagagggtgaagataggttgtctgaagcattataacttgtcttttaaaaaattcaatcataaatataaggaggtatgatgaagaaaaagattattagtgcaattttaatgtcaacggtcatcttaagcgctgctgccccattgtcaggtgtttatgcagcaaattttggtagattacattgtacaacagcagtaatacgtaatattaatgatcaagttttatttgttgataaaagacaacctgtttttgaagatatgactgatattgatcaatctgcatctgaaccacaaactagattaataatttatatgtataaagatagtgaagttagaggattagctgtaacattaagtgttaaagatagtaaaatgagtacattatcatgtaaaaacaaaataatttcatttgaagaaatggacccacctgaaaatattgatgatattcaatcagatttaattttctttcaaaaacgtgttccaggtcataacaaaatggaatttgaatctagtttatatgaaggtcactttttagcttgtcaaaaagaagatgatgcttttaaattaattttaaagaaaaaagatgaaaatggagataaatcagttatgtttacattaactaatttacatcaatcataataaacgcgtattaataaggaggctaactaatgaaaaagaaaatcatttcagcgattttgatgtcaacggttattttaagcgcagcagctccattatctggagtttatgcagccccaacacgtagtccaataacagtaactagaccttggaaacatgttgaagcaattaaagaagcattaaatttattagatgatatgccagtaacattaaatgaagaagttgaagtagtaagtaatgaatttagttttaaaaaattaacatgtgttcaaactagattaaaaatttttgaacaaggattaagaggtaattttactaaattaaaaggtgctttaaatatgacagctagttattatcaaacatattgtccaccaacacctgaaactgattgtgaaacacaagtaactacatatgctgattttattgattcattaaaaacatttttaactgatattccttttgaatgtaaaaaaccaggacaaaaataataaggcatgcggtaccactagttctagagagctcaagctttctttgaaccaaaattagaaaaccaaggcttgaaacgttcaattgaaatggcaattaaacaaattacagcacgtgttgctttgattgatagccaaaaagcagcagttgataaagcaattactgatattgctgaaaaattgtaatttataaataaaaatcaccttttagaggtggtttttttatttataaattattcgtttgatttcgctttcgatagaacaatcaaatcgtttctgagacgttttagcgtttatttcgtttagttatcggcataatcgttaaaacaggcgttatcgtagcgtaaaagcccttgagcgtagcgtggctttgcagcgaagatgttgtctgttagattatgaaagccgatgactgaatgaaataataagcgcagcgtccttctatttcggttggaggaggctcaagggagtttgagggaatgaaattccctcatgggtttgattttaaaaattgcttgcaattttgccgagcggtagcgctggaaaatttttgaaaaaaatttggaatttggaaaaaaatggggggaaaggaagcgaattttgcttccgtactacgaccccccattaagtgccgagtgccaatttttgtgccaaaaacgctctatcccaactggctcaagggtttgaggggtttttcaatcgccaacgaatcgccaacgttttcgccaacgttttttataaatctatatttaagtagctttatttttgtttttatgattacaaagtgatacactaattttataaaattatttgattggagttttttaaatggtgatttcagaatcgaaaaaaagagttatgatttctctgacaaaagagcaagataaaaaattaacagatatggcgaaacaaaaagatttttcaaaatctgcggttgcggcgttagctatagaagaatatgcaagaaaggaatcagaacaaaaaaaataagcgaaagctcgcgtttttagaaggatacgagttttcgctacttgtttttgataaggtaattatatcatggctattaaaaatactaaagctagaaattttggatttttattatatcctgactcaattcctaatgattggaaagaaaaattagagagtttgggcgtatctatggctgtcagtcctttacacgatatggacgaaaaaaaagataaagatacatggaatagtagtgatgttatacgaaatggaaagcactataaaaaaccacactatcacgttatatatattgcacgaaatcctgtaacaatagaaagcgttaggaacaagattaagcgaaaattggggaatagttcagttgctcatgttgagatacttgattatatcaaaggttcatatgaatatttgactcatgaatcaaaggacgctattgctaagaataaacatatatacgacaaaaaagatattttgaacattaatgattttgatattgaccgctatataacacttgatgaaagccaaaaaagagaattgaagaatttacttttagatatagtggatgactataatttggtaaatacaaaagatttaatggcttttattcgccttaggggagcggagtttggaattttaaatacgaatgatgtaaaagatattgtttcaacaaactctagcgcctttagattatggtttgagggcaattatcagtgtggatatagagcaagttatgcaaaggttcttgatgctgaaacgggggaaataaaatgacaaacaaagaaaaagagttatttgctgaaaatgaggaattaaaaaaagaaattaaggacttaaaagagcgtattgaaagatacagagaaatggaagttgaattaagtacaacaatagatttattgagaggagggattattgaataaataaaagcccccctgacgaaagtcgacatggtcgatgtctagatgcttaaactagagaaaggtttaaaagatgaaaacttcaccacatcgtaatacttcagctattgttgatttaaaagcgattagaaataatattgaaaaatttaaaaagcatattaaccctaatgcagagatttggccagcagtgaaagcagatgcttatggtcatggctcgattgaggtttctaaagcggtgagcgatttggtaggtggtttttgtgtatcaaacctagatgaggcaattgaattacgaaatcatctggtgactaaaccgattttagttttatccggaattgttccagaagatgttgatattgcagctgcccttaatattagtcttactgccccgagtttagaatggttgaaattggttgttcaagaagaagcagaactttcagatttaaaaattcatattggtgtagattctggtatgggtcggattggtattcgtgatgttgaagaagctaatcagatgattgaacttgctgataaatatgcgattaattttgaaggaattttcactcattttgcgactgcggatatggctgatgaaacaaaatttaaaaatcaacaggcaagatttaacaaaattatggccggattatcacgtcaaccaaaatttatacactcaactaatacggccgctgctttatggcataaggaacaagttcaagctattgaacgtttagggatttcaatgtatggcttgaatccaagtggtaaaactttggaacttccttttgaaattgaacccgctctctctttagtttctgaattgactcatataaaaaaaatagctgcaggtgaaacggttggttatggtgcaacttatgagacgagtgaagaaacttggattggaactgttccaattggttacgctgacgggtggacccgtcaaatgcaaggtttcaaagtgcttgttgatggaaagttttgtgagattgttggtcgagtttgtatggatcaaatgatgataaaacttgataagtcttaccctttgggaacgaaggtcactttgattggtcgagataaggctaatgaaatcacgacaacagacgttgctgattggcgtggaacgattaattatgaagtgctttgcttactttctgatagaatcaaaagaatctataaataaaattaaaaaaactgtatttttacagtttttttgttttctgttaaaagcagatgataacctcacta

SEQ ID NO: 24 - protein, 312 aa, Mus musculus
  mature form of mouse interleukin 12 (mIL-12) subunit beta
MWELEKDVYVVEVDWTPDAPGETVNLTCDTPEEDDITWTSDQRHGVIGSGKTLTITVKEFLDAGQYTCHKGGETLSHSHLLLHKKENGIWSTEILKNFKNKTFLKCEAPNYSGRFTCSWLVQRNMDLKFNIKSSSSSPDSRAVTCGMASLSAEKVTLDQRDYEKYSVSCQEDVTCPTAEETLPIELALEARQQNKYENYSTSFFIRDIIKPDPPKNLQMKPLKNSQVEVSWEYPDSWSTPHSYFSLKFFVRIQRKKEKMKETEEGCNQKGAFLVEKTSTEVQCKGGNVCVQAQDRYYNSSCSKWACVPCRVR

SEQ ID NO: 25 - protein, 193 aa, Mus musculus
  mature form of mouse interleukin 12 (mIL-12) subunit alpha isoform 2
RVIPVSGPARCLSQSRNLLKTTDDMVKTAREKLKHYSCTAEDIDHEDITRDQTSTLKTCLPLELHKNESCLATRETSSTTRGSCLPPQKTSLMMTLCLGSIYEDLKMYQTEFQAINAALQNHNHQQIILDKGMLVAIDELMQSLNHNGETLRQKPPVGEADPYRVKMKLCILLHAFSTRVVTINRVMGYLSSA

SEQ ID NO: 26 - protein, 523 aa, Artificial Sequence
  recombinant mIL-12 fusion protein
ADMWELEKDVYVVEVDWTPDAPGETVNLTCDTPEEDDITWTSDQRHGVIGSGKTLTITVKEFLDAGQYTCHKGGETLSHSHLLLHKKENGIWSTEILKNFKNKTFLKCEAPNYSGRFTCSWLVQRNMDLKFNIKSSSSSPDSRAVTCGMASLSAEKVTLDQRDYEKYSVSCQEDVTCPTAEETLPIELALEARQQNKYENYSTSFFIRDIIKPDPPKNLQMKPLKNSQVEVSWEYPDSWSTPHSYFSLKFFVRIQRKKEKMKETEEGCNQKGAFLVEKTSTEVQCKGGNVCVQAQDRYYNSSCSKWACVPCRVRSGGGGSGGGGSGGGGSRVIPVSGPARCLSQSRNLLKTTDDMVKTAREKLKHYSCTAEDIDHEDITRDQTSTLKTCLPLELHKNESCLATRETSSTTRGSCLPPQKTSLMMTLCLGSIYEDLKMYQTEFQAINAALQNHNHQQIILDKGMLVAIDELMQSLNHNGETLRQKPPVGEADPYRVKMKLCILLHAFSTRVVTINRVMGYLSSA

SEQ ID NO: 27 - protein, 550 aa, Artificial Sequence
  recombinant mIL-12 precursor protein
MKKKIISAILMSTVILSAAAPLSGVYAADMWELEKDVYVVEVDWTPDAPGETVNLTCDTPEEDDITWTSDQRHGVIGSGKTLTITVKEFLDAGQYTCHKGGETLSHSHLLLHKKENGIWSTEILKNFKNKTFLKCEAPNYSGRFTCSWLVQRNMDLKFNIKSSSSSPDSRAVTCGMASLSAEKVTLDQRDYEKYSVSCQEDVTCPTAEETLPIELALEARQQNKYENYSTSFFIRDIIKPDPPKNLQMKPLKNSQVEVSWEYPDSWSTPHSYFSLKFFVRIQRKKEKMKETEEGCNQKGAFLVEKTSTEVQCKGGNVCVQAQDRYYNSSCSKWACVPCRVRSGGGGSGGGGSGGGGSRVIPVSGPARCLSQSRNLLKTTDDMVKTAREKLKHYSCTAEDIDHEDITRDQTSTLKTCLPLELHKNESCLATRETSSTTRGSCLPPQKTSLMMTLCLGSIYEDLKMYQTEFQAINAALQNHNHQQIILDKGMLVAIDELMQSLNHNGETLRQKPPVGEADPYRVKMKLCILLHAFSTRVVTINRVMGYLSSA

SEQ ID NO: 28 - protein, 168 aa, Mus musculus
  mature form of mouse interferon alpha-2 (mIFNa2)
GCDLPHTYNLRNKRALKVLAQMRRLPFLSCLKDRQDFGFPLEKVDNQQIQKAQAIPVLRDLTQQTLNLFTSKASSAAWNTTLLDSFCNDLHQQLNDLQTCLMQQVGVQEPPLTQEDALLAVRKYFHRITVYLREKKHSPCAWEVVRAEVWRALSSSVNLLPRLSEEKE

SEQ ID NO: 29 - protein, 169 aa, Artificial Sequence
  recombinant variant of mIFNa2
AGCDLPHTYNLRNKRALKVLAQMRRLPFLSCLKDRQDFGFPLEKVDNQQIQKAQAIPVLRDLTQQTLNLFTSKASSAAWNTTLLDSFCNDLHQQLNDLQTCLMQQVGVQEPPLTQEDALLAVRKYFHRITVYLREKKHSPCAWEVVRAEVWRALSSSVNLLPRLSEEKE

SEQ ID NO: 30 - protein, 196 aa, Artificial Sequence
  recombinant mIFNa2 precursor protein
MKKKIISAILMSTVILSAAAPLSGVYAAGCDLPHTYNLRNKRALKVLAQMRRLPFLSCLKDRQDFGFPLEKVDNQQIQKAQAIPVLRDLTQQTLNLFTSKASSAAWNTTLLDSFCNDLHQQLNDLQTCLMQQVGVQEPPLTQEDALLAVRKYFHRITVYLREKKHSPCAWEVVRAEVWRALSSSVNLLPRLSEEKE

SEQ ID NO: 31 - DNA, 4135 bp, Artificial Sequence
  synthetic mTEA construct
agatctgagcgttgtataagcttttatgtctttctatatcaacttttaatagaaatataaagtaatataaatgtttttataataaattatgtgagatatatttttttgtccgtactggtatagatttgacgattaagtcttaaataagttataatctcaattgcgtaatttcttaaatacagaaataacaactacattggtagactgattaaaaagtgtacttgatgaactgttataaaccttaaaaaaataaaaataatagtttgggggatgttaaagatgtataaaaaatatggagattgttttaaaaagttgcgaaaccaaaagaatttagggttatcatactttagtaaacttggaatagaccgttcaaatatatctagatttgaacatggaaaatgtatgatgagttttgagcgtatagatttgatgttagaagaaatgcaagttccgttatctgagtacgaattgattgtaaataattttatgccgaatttccaagaattttttatattagaattggaaaaagctgaatttagccaaaatcgagataaaataaaagagttgtattctgaggtcaaagaaacggggaatcatttactgacggttaccgtgaaaacgaagcttgggaatataagtcagacagaagttaaagaaattgaagcttatctttgcaatattgaagagtggggatattttgaacttactttattttattttgtatctgattatctcaatgtcaatcaattagaattgctgctttttaattttgataaaagatgtgaaaattactgtagagtcttaaaatatagaaggagactattgcaaatagcctataaaagtgttgcgatatacgcggctaaaggagaaagaaaaaaagccgaaaatattttagaaatgactaaaaaatatcgaactgtgggagtcgatttatattcagaagtattaagacatcttgctagagctatcattatttttaattttgaaaatgcagagattggggaagaaaaaataaattatgctcttgagattttggaagaatttggaggaaagaagataaaagaattctatcagaataaaatggaaaagtatttgaaaaggtcaatttagtctcttttgagctgttgctttaaagcaacagctcaaaagagattttctttattctagagcatatactagagggtgaagataggttgtctgaagcattataacttgtcttttaaaaaattcaatcataaatataaggaggtatgatgaagaaaaagattattagtgcaattttaatgtcaacggtcatcttaagcgctgctgccccattgtcaggtgtttatgcagccgatatgtgggaattagaaaaagatgtttatgttgtagaagttgattggacaccagatgctcctggtgaaacagttaatttaacatgtgatactccagaagaagatgatattacatggacatctgatcaacgacatggagttattggtagtggaaaaacattaacaattacagttaaagaatttttagatgctggacaatatacttgtcataaaggaggtgaaacattatctcattcacatttattattacataaaaaagaaaatggtatttggtcaactgaaatcttaaaaaattttaaaaataagacatttttaaaatgtgaagctcctaattattctggtagatttacttgttcatggttagttcaaagaaatatggatttaaaatttaatattaaatcaagttcaagtagtcctgatagtagagctgtaacatgtggaatggcaagtttatctgctgaaaaagtaacacttgatcaacgtgattatgaaaaatattctgttagttgtcaagaagatgttacttgtccaacagctgaagaaacattaccaattgaattagcattagaagctagacaacaaaacaaatatgaaaattatagtacatctttctttattcgtgacattattaaacctgatccacctaaaaatttacaaatgaaacctttaaaaaatagtcaagttgaagttagttgggaatatccagattcatggtcaacaccacattcatatttttcattaaaattctttgttagaattcaacgtaaaaaagaaaaaatgaaagaaactgaagaaggttgtaaccaaaaaggtgcatttttagttgaaaaaactagtactgaagttcaatgtaaaggtggtaatgtatgtgttcaagctcaagatcgatattataattctagttgttcaaaatgggcatgtgttccatgtagagttcgtagtggaggaggtggaagtggtggaggtggttcaggtggtggaggttcacgtgtaattccagtttcaggacctgctcgatgtttaagtcaatctcgaaatttattaaaaactacagatgatatggttaaaactgctagagaaaaattaaaacattatagttgtacagctgaagatattgatcatgaagatattacacgtgatcaaacttcaacacttaaaacatgtttaccacttgaattacataaaaatgaatcttgtttagctactagagaaactagtagtacaactagaggttcttgtttgcctccacaaaaaacatcattaatgatgacattatgtttaggttctatttatgaagatttgaaaatgtatcaaactgaatttcaagcaattaatgctgctttacaaaatcataatcatcaacaaattattttagataaaggtatgttagttgcaattgatgaattaatgcaatctttaaatcataatggtgaaactcttagacaaaaaccacctgttggagaagcagacccttatcgagtgaaaatgaaattatgtatcttgttgcacgctttttcaacacgggtagtcacaattaatcgtgtaatgggatatttgagtagtgcataataaacgcgtattaataaggaggctaactaatgaaaaagaaaatcatttcagcgattttgatgtcaacggttattttaagcgcagcagctccattatctggagtttatgcagcaaattttggtagattacattgtacaacagcagtaatacgtaatattaatgatcaagttttatttgttgataaaagacaacctgtttttgaagatatgactgatattgatcaatctgcatctgaaccacaaactagattaataatttatatgtataaagatagtgaagttagaggattagctgtaacattaagtgttaaagatagtaaaatgagtacattatcatgtaaaaacaaaataatttcatttgaagaaatggacccacctgaaaatattgatgatattcaatcagatttaattttctttcaaaaacgtgttccaggtcataacaaaatggaatttgaatctagtttatatgaaggtcactttttagcttgtcaaaaagaagatgatgcttttaaattaattttaaagaaaaaagatgaaaatggagataaatcagttatgtttacattaactaatttacatcaatcataataaacgcgtgaaatttaggaggtagtccaaatgaaaaaaaagattatctcagctattttaatgtctacagtgatactttctgctgcagccccgttgtcaggtgtttacgctgcctgtgatttaccacatacttataatttaagaaataagcgtgctttaaaagttttagcacaaatgagacgtttaccatttttaagttgtttaaaagatagacaagattttggttttccattagaaaaagtagataatcaacaaattcaaaaagctcaagcaattcctgttttaagagatttaacacaacaaacattaaatttatttactagtaaagctagtagtgcagcttggaatgcaacattattagatagtttttgtaatgatttacatcaacaattaaatgatttacaaacatgtttaatgcaacaagtaggagttcaagaacctccattaactcaagaagatgcattattagctgttagaaaatattttcatagaataaccgtttatttaagagaaaagaaacatagtccttgtgcttgggaagtagttagagctgaagtttggagagctttaagttcatcagttaatttattacctagattaagtgaagaaaaagaataataaccatgggtactgcaggcatgc

SEQ ID NO: 32 - DNA, 7261 bp, Artificial Sequence
  plasmid pC-mTEA
gatctgagcgttgtataagcttttatgtctttctatatcaacttttaatagaaatataaagtaatataaatgtttttataataaattatgtgagatatatttttttgtccgtactggtatagatttgacgattaagtcttaaataagttataatctcaattgcgtaatttcttaaatacagaaataacaactacattggtagactgattaaaaagtgtacttgatgaactgttataaaccttaaaaaaataaaaataatagtttgggggatgttaaagatgtataaaaaatatggagattgttttaaaaagttgcgaaaccaaaagaatttagggttatcatactttagtaaacttggaatagaccgttcaaatatatctagatttgaacatggaaaatgtatgatgagttttgagcgtatagatttgatgttagaagaaatgcaagttccgttatctgagtacgaattgattgtaaataattttatgccgaatttccaagaattttttatattagaattggaaaaagctgaatttagccaaaatcgagataaaataaaagagttgtattctgaggtcaaagaaacggggaatcatttactgacggttaccgtgaaaacgaagcttgggaatataagtcagacagaagttaaagaaattgaagcttatctttgcaatattgaagagtggggatattttgaacttactttattttattttgtatctgattatctcaatgtcaatcaattagaattgctgctttttaattttgataaaagatgtgaaaattactgtagagtcttaaaatatagaaggagactattgcaaatagcctataaaagtgttgcgatatacgcggctaaaggagaaagaaaaaaagccgaaaatattttagaaatgactaaaaaatatcgaactgtgggagtcgatttatattcagaagtattaagacatcttgctagagctatcattatttttaattttgaaaatgcagagattggggaagaaaaaataaattatgctcttgagattttggaagaatttggaggaaagaagataaaagaattctatcagaataaaatggaaaagtatttgaaaaggtcaatttagtctcttttgagctgttgctttaaagcaacagctcaaaagagattttctttattctagagcatatactagagggtgaagataggttgtctgaagcattataacttgtcttttaaaaaattcaatcataaatataaggaggtatgatgaagaaaaagattattagtgcaattttaatgtcaacggtcatcttaagcgctgctgccccattgtcaggtgtttatgcagccgatatgtgggaattagaaaaagatgtttatgttgtagaagttgattggacaccagatgctcctggtgaaacagttaatttaacatgtgatactccagaagaagatgatattacatggacatctgatcaacgacatggagttattggtagtggaaaaacattaacaattacagttaaagaatttttagatgctggacaatatacttgtcataaaggaggtgaaacattatctcattcacatttattattacataaaaaagaaaatggtatttggtcaactgaaatcttaaaaaattttaaaaataagacatttttaaaatgtgaagctcctaattattctggtagatttacttgttcatggttagttcaaagaaatatggatttaaaatttaatattaaatcaagttcaagtagtcctgatagtagagctgtaacatgtggaatggcaagtttatctgctgaaaaagtaacacttgatcaacgtgattatgaaaaatattctgttagttgtcaagaagatgttacttgtccaacagctgaagaaacattaccaattgaattagcattagaagctagacaacaaaacaaatatgaaaattatagtacatctttctttattcgtgacattattaaacctgatccacctaaaaatttacaaatgaaacctttaaaaaatagtcaagttgaagttagttgggaatatccagattcatggtcaacaccacattcatatttttcattaaaattctttgttagaattcaacgtaaaaaagaaaaaatgaaagaaactgaagaaggttgtaaccaaaaaggtgcatttttagttgaaaaaactagtactgaagttcaatgtaaaggtggtaatgtatgtgttcaagctcaagatcgatattataattctagttgttcaaaatgggcatgtgttccatgtagagttcgtagtggaggaggtggaagtggtggaggtggttcaggtggtggaggttcacgtgtaattccagtttcaggacctgctcgatgtttaagtcaatctcgaaatttattaaaaactacagatgatatggttaaaactgctagagaaaaattaaaacattatagttgtacagctgaagatattgatcatgaagatattacacgtgatcaaacttcaacacttaaaacatgtttaccacttgaattacataaaaatgaatcttgtttagctactagagaaactagtagtacaactagaggttcttgtttgcctccacaaaaaacatcattaatgatgacattatgtttaggttctatttatgaagatttgaaaatgtatcaaactgaatttcaagcaattaatgctgctttacaaaatcataatcatcaacaaattattttagataaaggtatgttagttgcaattgatgaattaatgcaatctttaaatcataatggtgaaactcttagacaaaaaccacctgttggagaagcagacccttatcgagtgaaaatgaaattatgtatcttgttgcacgctttttcaacacgggtagtcacaattaatcgtgtaatgggatatttgagtagtgcataataaacgcgtattaataaggaggctaactaatgaaaaagaaaatcatttcagcgattttgatgtcaacggttattttaagcgcagcagctccattatctggagtttatgcagcaaattttggtagattacattgtacaacagcagtaatacgtaatattaatgatcaagttttatttgttgataaaagacaacctgtttttgaagatatgactgatattgatcaatctgcatctgaaccacaaactagattaataatttatatgtataaagatagtgaagttagaggattagctgtaacattaagtgttaaagatagtaaaatgagtacattatcatgtaaaaacaaaataatttcatttgaagaaatggacccacctgaaaatattgatgatattcaatcagatttaattttctttcaaaaacgtgttccaggtcataacaaaatggaatttgaatctagtttatatgaaggtcactttttagcttgtcaaaaagaagatgatgcttttaaattaattttaaagaaaaaagatgaaaatggagataaatcagttatgtttacattaactaatttacatcaatcataataaacgcgtgaaatttaggaggtagtccaaatgaaaaaaaagattatctcagctattttaatgtctacagtgatactttctgctgcagccccgttgtcaggtgtttacgctgcctgtgatttaccacatacttataatttaagaaataagcgtgctttaaaagttttagcacaaatgagacgtttaccatttttaagttgtttaaaagatagacaagattttggttttccattagaaaaagtagataatcaacaaattcaaaaagctcaagcaattcctgttttaagagatttaacacaacaaacattaaatttatttactagtaaagctagtagtgcagcttggaatgcaacattattagatagtttttgtaatgatttacatcaacaattaaatgatttacaaacatgtttaatgcaacaagtaggagttcaagaacctccattaactcaagaagatgcattattagctgttagaaaatattttcatagaataaccgtttatttaagagaaaagaaacatagtccttgtgcttgggaagtagttagagctgaagtttggagagctttaagttcatcagttaatttattacctagattaagtgaagaaaaagaataataaccatgggtactgcaggcatgcggtaccactagttctagagagctcaagctttctttgaaccaaaattagaaaaccaaggcttgaaacgttcaattgaaatggcaattaaacaaattacagcacgtgttgctttgattgatagccaaaaagcagcagttgataaagcaattactgatattgctgaaaaattgtaatttataaataaaaatcaccttttagaggtggtttttttatttataaattattcgtttgatttcgctttcgatagaacaatcaaatcgtttctgagacgttttagcgtttatttcgtttagttatcggcataatcgttaaaacaggcgttatcgtagcgtaaaagcccttgagcgtagcgtggctttgcagcgaagatgttgtctgttagattatgaaagccgatgactgaatgaaataataagcgcagcgtccttctatttcggttggaggaggctcaagggagtttgagggaatgaaattccctcatgggtttgattttaaaaattgcttgcaattttgccgagcggtagcgctggaaaatttttgaaaaaaatttggaatttggaaaaaaatggggggaaaggaagcgaattttgcttccgtactacgaccccccattaagtgccgagtgccaatttttgtgccaaaaacgctctatcccaactggctcaagggtttgaggggtttttcaatcgccaacgaatcgccaacgttttcgccaacgttttttataaatctatatttaagtagctttatttttgtttttatgattacaaagtgatacactaattttataaaattatttgattggagttttttaaatggtgatttcagaatcgaaaaaaagagttatgatttctctgacaaaagagcaagataaaaaattaacagatatggcgaaacaaaaagatttttcaaaatctgcggttgcggcgttagctatagaagaatatgcaagaaaggaatcagaacaaaaaaaataagcgaaagctcgcgtttttagaaggatacgagttttcgctacttgtttttgataaggtaattatatcatggctattaaaaatactaaagctagaaattttggatttttattatatcctgactcaattcctaatgattggaaagaaaaattagagagtttgggcgtatctatggctgtcagtcctttacacgatatggacgaaaaaaaagataaagatacatggaatagtagtgatgttatacgaaatggaaagcactataaaaaaccacactatcacgttatatatattgcacgaaatcctgtaacaatagaaagcgttaggaacaagattaagcgaaaattggggaatagttcagttgctcatgttgagatacttgattatatcaaaggttcatatgaatatttgactcatgaatcaaaggacgctattgctaagaataaacatatatacgacaaaaaagatattttgaacattaatgattttgatattgaccgctatataacacttgatgaaagccaaaaaagagaattgaagaatttacttttagatatagtggatgactataatttggtaaatacaaaagatttaatggcttttattcgccttaggggagcggagtttggaattttaaatacgaatgatgtaaaagatattgtttcaacaaactctagcgcctttagattatggtttgagggcaattatcagtgtggatatagagcaagttatgcaaaggttcttgatgctgaaacgggggaaataaaatgacaaacaaagaaaaagagttatttgctgaaaatgaggaattaaaaaaagaaattaaggacttaaaagagcgtattgaaagatacagagaaatggaagttgaattaagtacaacaatagatttattgagaggagggattattgaataaataaaagcccccctgacgaaagtcgacatggtcgatgtctagatgcttaaactagagaaaggtttaaaagatgaaaacttcaccacatcgtaatacttcagctattgttgatttaaaagcgattagaaataatattgaaaaatttaaaaagcatattaaccctaatgcagagatttggccagcagtgaaagcagatgcttatggtcatggctcgattgaggtttctaaagcggtgagcgatttggtaggtggtttttgtgtatcaaacctagatgaggcaattgaattacgaaatcatctggtgactaaaccgattttagttttatccggaattgttccagaagatgttgatattgcagctgcccttaatattagtcttactgccccgagtttagaatggttgaaattggttgttcaagaagaagcagaactttcagatttaaaaattcatattggtgtagattctggtatgggtcggattggtattcgtgatgttgaagaagctaatcagatgattgaacttgctgataaatatgcgattaattttgaaggaattttcactcattttgcgactgcggatatggctgatgaaacaaaatttaaaaatcaacaggcaagatttaacaaaattatggccggattatcacgtcaaccaaaatttatacactcaactaatacggccgctgctttatggcataaggaacaagttcaagctattgaacgtttagggatttcaatgtatggcttgaatccaagtggtaaaactttggaacttccttttgaaattgaacccgctctctctttagtttctgaattgactcatataaaaaaaatagctgcaggtgaaacggttggttatggtgcaacttatgagacgagtgaagaaacttggattggaactgttccaattggttacgctgacgggtggacccgtcaaatgcaaggtttcaaagtgcttgttgatggaaagttttgtgagattgttggtcgagtttgtatggatcaaatgatgataaaacttgataagtcttaccctttgggaacgaaggtcactttgattggtcgagataaggctaatgaaatcacgacaacagacgttgctgattggcgtggaacgattaattatgaagtgctttgcttactttctgatagaatcaaaagaatctataaataaaattaaaaaaactgtatttttacagtttttttgttttctgttaaaagcagatgataacctcacta

SEQ ID NO: 33 - DNA, 4003 bp, Artificial Sequence
  synthetic mGTE construct
agatctgagcgttgtataagcttttatgtctttctatatcaacttttaatagaaatataaagtaatataaatgtttttataataaattatgtgagatatatttttttgtccgtactggtatagatttgacgattaagtcttaaataagttataatctcaattgcgtaatttcttaaatacagaaataacaactacattggtagactgattaaaaagtgtacttgatgaactgttataaaccttaaaaaaataaaaataatagtttgggggatgttaaagatgtataaaaaatatggagattgttttaaaaagttgcgaaaccaaaagaatttagggttatcatactttagtaaacttggaatagaccgttcaaatatatctagatttgaacatggaaaatgtatgatgagttttgagcgtatagatttgatgttagaagaaatgcaagttccgttatctgagtacgaattgattgtaaataattttatgccgaatttccaagaattttttatattagaattggaaaaagctgaatttagccaaaatcgagataaaataaaagagttgtattctgaggtcaaagaaacggggaatcatttactgacggttaccgtgaaaacgaagcttgggaatataagtcagacagaagttaaagaaattgaagcttatctttgcaatattgaagagtggggatattttgaacttactttattttattttgtatctgattatctcaatgtcaatcaattagaattgctgctttttaattttgataaaagatgtgaaaattactgtagagtcttaaaatatagaaggagactattgcaaatagcctataaaagtgttgcgatatacgcggctaaaggagaaagaaaaaaagccgaaaatattttagaaatgactaaaaaatatcgaactgtgggagtcgatttatattcagaagtattaagacatcttgctagagctatcattatttttaattttgaaaatgcagagattggggaagaaaaaataaattatgctcttgagattttggaagaatttggaggaaagaagataaaagaattctatcagaataaaatggaaaagtatttgaaaaggtcaatttagtctcttttgagctgttgctttaaagcaacagctcaaaagagattttctttattctagagcatatactagagggtgaagataggttgtctgaagcattataacttgtcttttaaaaaattcaatcataaatataaggaggtatgatgaagaaaaagattattagtgcaattttaatgtcaacggtcatcttaagcgctgctgccccattgtcaggtgtttatgcagccccaacacgtagtccaataacagtaactagaccttggaaacatgttgaagcaattaaagaagcattaaatttattagatgatatgccagtaacattaaatgaagaagttgaagtagtaagtaatgaatttagttttaaaaaattaacatgtgttcaaactagattaaaaatttttgaacaaggattaagaggtaattttactaaattaaaaggtgctttaaatatgacagctagttattatcaaacatattgtccaccaacacctgaaactgattgtgaaacacaagtaactacatatgctgattttattgattcattaaaaacatttttaactgatattccttttgaatgtaaaaaaccaggacaaaaataataaacgcgtattaataaggaggctaactaatgaaaaagaaaatcatttcagcgattttgatgtcaacggttattttaagcgcagcagctccattatctggagtttatgcagccgatatgtgggaattagaaaaagatgtttatgttgtagaagttgattggacaccagatgctcctggtgaaacagttaatttaacatgtgatactccagaagaagatgatattacatggacatctgatcaacgacatggagttattggtagtggaaaaacattaacaattacagttaaagaatttttagatgctggacaatatacttgtcataaaggaggtgaaacattatctcattcacatttattattacataaaaaagaaaatggtatttggtcaactgaaatcttaaaaaattttaaaaataagacatttttaaaatgtgaagctcctaattattctggtagatttacttgttcatggttagttcaaagaaatatggatttaaaatttaatattaaatcaagttcaagtagtcctgatagtagagctgtaacatgtggaatggcaagtttatctgctgaaaaagtaacacttgatcaacgtgattatgaaaaatattctgttagttgtcaagaagatgttacttgtccaacagctgaagaaacattaccaattgaattagcattagaagctagacaacaaaacaaatatgaaaattatagtacatctttctttattcgtgacattattaaacctgatccacctaaaaatttacaaatgaaacctttaaaaaatagtcaagttgaagttagttgggaatatccagattcatggtcaacaccacattcatatttttcattaaaattctttgttagaattcaacgtaaaaaagaaaaaatgaaagaaactgaagaaggttgtaaccaaaaaggtgcatttttagttgaaaaaactagtactgaagttcaatgtaaaggtggtaatgtatgtgttcaagctcaagatcgatattataattctagttgttcaaaatgggcatgtgttccatgtagagttcgtagtggaggaggtggaagtggtggaggtggttcaggtggtggaggttcacgtgtaattccagtttcaggacctgctcgatgtttaagtcaatctcgaaatttattaaaaactacagatgatatggttaaaactgctagagaaaaattaaaacattatagttgtacagctgaagatattgatcatgaagatattacacgtgatcaaacttcaacacttaaaacatgtttaccacttgaattacataaaaatgaatcttgtttagctactagagaaactagtagtacaactagaggttcttgtttgcctccacaaaaaacatcattaatgatgacattatgtttaggttctatttatgaagatttgaaaatgtatcaaactgaatttcaagcaattaatgctgctttacaaaatcataatcatcaacaaattattttagataaaggtatgttagttgcaattgatgaattaatgcaatctttaaatcataatggtgaaactcttagacaaaaaccacctgttggagaagcagacccttatcgagtgaaaatgaaattatgtatcttgttgcacgctttttcaacacgggtagtcacaattaatcgtgtaatgggatatttgagtagtgcataataaacgcgtgaaatttaggaggtagtccaaatgaaaaaaaagattatctcagctattttaatgtctacagtgatactttctgctgcagccccgttgtcaggtgtttacgctgcaaattttggtagattacattgtacaacagcagtaatacgtaatattaatgatcaagttttatttgttgataaaagacaacctgtttttgaagatatgactgatattgatcaatctgcatctgaaccacaaactagattaataatttatatgtataaagatagtgaagttagaggattagctgtaacattaagtgttaaagatagtaaaatgagtacattatcatgtaaaaacaaaataatttcatttgaagaaatggacccacctgaaaatattgatgatattcaatcagatttaattttctttcaaaaacgtgttccaggtcataacaaaatggaatttgaatctagtttatatgaaggtcactttttagcttgtcaaaaagaagatgatgcttttaaattaattttaaagaaaaaagatgaaaatggagataaatcagttatgtttacattaactaatttacatcaatcataataaccatgggtactgcaggcatgc

SEQ ID NO: 34 - DNA, 7129 bp, Artificial Sequence
  plasmid pC-mGTE
gatctgagcgttgtataagcttttatgtctttctatatcaacttttaatagaaatataaagtaatataaatgtttttataataaattatgtgagatatatttttttgtccgtactggtatagatttgacgattaagtcttaaataagttataatctcaattgcgtaatttcttaaatacagaaataacaactacattggtagactgattaaaaagtgtacttgatgaactgttataaaccttaaaaaaataaaaataatagtttgggggatgttaaagatgtataaaaaatatggagattgttttaaaaagttgcgaaaccaaaagaatttagggttatcatactttagtaaacttggaatagaccgttcaaatatatctagatttgaacatggaaaatgtatgatgagttttgagcgtatagatttgatgttagaagaaatgcaagttccgttatctgagtacgaattgattgtaaataattttatgccgaatttccaagaattttttatattagaattggaaaaagctgaatttagccaaaatcgagataaaataaaagagttgtattctgaggtcaaagaaacggggaatcatttactgacggttaccgtgaaaacgaagcttgggaatataagtcagacagaagttaaagaaattgaagcttatctttgcaatattgaagagtggggatattttgaacttactttattttattttgtatctgattatctcaatgtcaatcaattagaattgctgctttttaattttgataaaagatgtgaaaattactgtagagtcttaaaatatagaaggagactattgcaaatagcctataaaagtgttgcgatatacgcggctaaaggagaaagaaaaaaagccgaaaatattttagaaatgactaaaaaatatcgaactgtgggagtcgatttatattcagaagtattaagacatcttgctagagctatcattatttttaattttgaaaatgcagagattggggaagaaaaaataaattatgctcttgagattttggaagaatttggaggaaagaagataaaagaattctatcagaataaaatggaaaagtatttgaaaaggtcaatttagtctcttttgagctgttgctttaaagcaacagctcaaaagagattttctttattctagagcatatactagagggtgaagataggttgtctgaagcattataacttgtcttttaaaaaattcaatcataaatataaggaggtatgatgaagaaaaagattattagtgcaattttaatgtcaacggtcatcttaagcgctgctgccccattgtcaggtgtttatgcagccccaacacgtagtccaataacagtaactagaccttggaaacatgttgaagcaattaaagaagcattaaatttattagatgatatgccagtaacattaaatgaagaagttgaagtagtaagtaatgaatttagttttaaaaaattaacatgtgttcaaactagattaaaaatttttgaacaaggattaagaggtaattttactaaattaaaaggtgctttaaatatgacagctagttattatcaaacatattgtccaccaacacctgaaactgattgtgaaacacaagtaactacatatgctgattttattgattcattaaaaacatttttaactgatattccttttgaatgtaaaaaaccaggacaaaaataataaacgcgtattaataaggaggctaactaatgaaaaagaaaatcatttcagcgattttgatgtcaacggttattttaagcgcagcagctccattatctggagtttatgcagccgatatgtgggaattagaaaaagatgtttatgttgtagaagttgattggacaccagatgctcctggtgaaacagttaatttaacatgtgatactccagaagaagatgatattacatggacatctgatcaacgacatggagttattggtagtggaaaaacattaacaattacagttaaagaatttttagatgctggacaatatacttgtcataaaggaggtgaaacattatctcattcacatttattattacataaaaaagaaaatggtatttggtcaactgaaatcttaaaaaattttaaaaataagacatttttaaaatgtgaagctcctaattattctggtagatttacttgttcatggttagttcaaagaaatatggatttaaaatttaatattaaatcaagttcaagtagtcctgatagtagagctgtaacatgtggaatggcaagtttatctgctgaaaaagtaacacttgatcaacgtgattatgaaaaatattctgttagttgtcaagaagatgttacttgtccaacagctgaagaaacattaccaattgaattagcattagaagctagacaacaaaacaaatatgaaaattatagtacatctttctttattcgtgacattattaaacctgatccacctaaaaatttacaaatgaaacctttaaaaaatagtcaagttgaagttagttgggaatatccagattcatggtcaacaccacattcatatttttcattaaaattctttgttagaattcaacgtaaaaaagaaaaaatgaaagaaactgaagaaggttgtaaccaaaaaggtgcatttttagttgaaaaaactagtactgaagttcaatgtaaaggtggtaatgtatgtgttcaagctcaagatcgatattataattctagttgttcaaaatgggcatgtgttccatgtagagttcgtagtggaggaggtggaagtggtggaggtggttcaggtggtggaggttcacgtgtaattccagtttcaggacctgctcgatgtttaagtcaatctcgaaatttattaaaaactacagatgatatggttaaaactgctagagaaaaattaaaacattatagttgtacagctgaagatattgatcatgaagatattacacgtgatcaaacttcaacacttaaaacatgtttaccacttgaattacataaaaatgaatcttgtttagctactagagaaactagtagtacaactagaggttcttgtttgcctccacaaaaaacatcattaatgatgacattatgtttaggttctatttatgaagatttgaaaatgtatcaaactgaatttcaagcaattaatgctgctttacaaaatcataatcatcaacaaattattttagataaaggtatgttagttgcaattgatgaattaatgcaatctttaaatcataatggtgaaactcttagacaaaaaccacctgttggagaagcagacccttatcgagtgaaaatgaaattatgtatcttgttgcacgctttttcaacacgggtagtcacaattaatcgtgtaatgggatatttgagtagtgcataataaacgcgtgaaatttaggaggtagtccaaatgaaaaaaaagattatctcagctattttaatgtctacagtgatactttctgctgcagccccgttgtcaggtgtttacgctgcaaattttggtagattacattgtacaacagcagtaatacgtaatattaatgatcaagttttatttgttgataaaagacaacctgtttttgaagatatgactgatattgatcaatctgcatctgaaccacaaactagattaataatttatatgtataaagatagtgaagttagaggattagctgtaacattaagtgttaaagatagtaaaatgagtacattatcatgtaaaaacaaaataatttcatttgaagaaatggacccacctgaaaatattgatgatattcaatcagatttaattttctttcaaaaacgtgttccaggtcataacaaaatggaatttgaatctagtttatatgaaggtcactttttagcttgtcaaaaagaagatgatgcttttaaattaattttaaagaaaaaagatgaaaatggagataaatcagttatgtttacattaactaatttacatcaatcataataaccatgggtactgcaggcatgcggtaccactagttctagagagctcaagctttctttgaaccaaaattagaaaaccaaggcttgaaacgttcaattgaaatggcaattaaacaaattacagcacgtgttgctttgattgatagccaaaaagcagcagttgataaagcaattactgatattgctgaaaaattgtaatttataaataaaaatcaccttttagaggtggtttttttatttataaattattcgtttgatttcgctttcgatagaacaatcaaatcgtttctgagacgttttagcgtttatttcgtttagttatcggcataatcgttaaaacaggcgttatcgtagcgtaaaagcccttgagcgtagcgtggctttgcagcgaagatgttgtctgttagattatgaaagccgatgactgaatgaaataataagcgcagcgtccttctatttcggttggaggaggctcaagggagtttgagggaatgaaattccctcatgggtttgattttaaaaattgcttgcaattttgccgagcggtagcgctggaaaatttttgaaaaaaatttggaatttggaaaaaaatggggggaaaggaagcgaattttgcttccgtactacgaccccccattaagtgccgagtgccaatttttgtgccaaaaacgctctatcccaactggctcaagggtttgaggggtttttcaatcgccaacgaatcgccaacgttttcgccaacgttttttataaatctatatttaagtagctttatttttgtttttatgattacaaagtgatacactaattttataaaattatttgattggagttttttaaatggtgatttcagaatcgaaaaaaagagttatgatttctctgacaaaagagcaagataaaaaattaacagatatggcgaaacaaaaagatttttcaaaatctgcggttgcggcgttagctatagaagaatatgcaagaaaggaatcagaacaaaaaaaataagcgaaagctcgcgtttttagaaggatacgagttttcgctacttgtttttgataaggtaattatatcatggctattaaaaatactaaagctagaaattttggatttttattatatcctgactcaattcctaatgattggaaagaaaaattagagagtttgggcgtatctatggctgtcagtcctttacacgatatggacgaaaaaaaagataaagatacatggaatagtagtgatgttatacgaaatggaaagcactataaaaaaccacactatcacgttatatatattgcacgaaatcctgtaacaatagaaagcgttaggaacaagattaagcgaaaattggggaatagttcagttgctcatgttgagatacttgattatatcaaaggttcatatgaatatttgactcatgaatcaaaggacgctattgctaagaataaacatatatacgacaaaaaagatattttgaacattaatgattttgatattgaccgctatataacacttgatgaaagccaaaaaagagaattgaagaatttacttttagatatagtggatgactataatttggtaaatacaaaagatttaatggcttttattcgccttaggggagcggagtttggaattttaaatacgaatgatgtaaaagatattgtttcaacaaactctagcgcctttagattatggtttgagggcaattatcagtgtggatatagagcaagttatgcaaaggttcttgatgctgaaacgggggaaataaaatgacaaacaaagaaaaagagttatttgctgaaaatgaggaattaaaaaaagaaattaaggacttaaaagagcgtattgaaagatacagagaaatggaagttgaattaagtacaacaatagatttattgagaggagggattattgaataaataaaagcccccctgacgaaagtcgacatggtcgatgtctagatgcttaaactagagaaaggtttaaaagatgaaaacttcaccacatcgtaatacttcagctattgttgatttaaaagcgattagaaataatattgaaaaatttaaaaagcatattaaccctaatgcagagatttggccagcagtgaaagcagatgcttatggtcatggctcgattgaggtttctaaagcggtgagcgatttggtaggtggtttttgtgtatcaaacctagatgaggcaattgaattacgaaatcatctggtgactaaaccgattttagttttatccggaattgttccagaagatgttgatattgcagctgcccttaatattagtcttactgccccgagtttagaatggttgaaattggttgttcaagaagaagcagaactttcagatttaaaaattcatattggtgtagattctggtatgggtcggattggtattcgtgatgttgaagaagctaatcagatgattgaacttgctgataaatatgcgattaattttgaaggaattttcactcattttgcgactgcggatatggctgatgaaacaaaatttaaaaatcaacaggcaagatttaacaaaattatggccggattatcacgtcaaccaaaatttatacactcaactaatacggccgctgctttatggcataaggaacaagttcaagctattgaacgtttagggatttcaatgtatggcttgaatccaagtggtaaaactttggaacttccttttgaaattgaacccgctctctctttagtttctgaattgactcatataaaaaaaatagctgcaggtgaaacggttggttatggtgcaacttatgagacgagtgaagaaacttggattggaactgttccaattggttacgctgacgggtggacccgtcaaatgcaaggtttcaaagtgcttgttgatggaaagttttgtgagattgttggtcgagtttgtatggatcaaatgatgataaaacttgataagtcttaccctttgggaacgaaggtcactttgattggtcgagataaggctaatgaaatcacgacaacagacgttgctgattggcgtggaacgattaattatgaagtgctttgcttactttctgatagaatcaaaagaatctataaataaaattaaaaaaactgtatttttacagtttttttgttttctgttaaaagcagatgataacctcacta

SEQ ID NO: 35 - DNA, 1970 bp, Artificial Sequence
  synthetic mCherry construct
agatctgagcgttgtataagcttttatgtctttctatatcaacttttaatagaaatataaagtaatataaatgtttttataataaattatgtgagatatatttttttgtccgtactggtatagatttgacgattaagtcttaaataagttataatctcaattgcgtaatttcttaaatacagaaataacaactacattggtagactgattaaaaagtgtacttgatgaactgttataaaccttaaaaaaataaaaataatagtttgggggatgttaaagatgtataaaaaatatggagattgttttaaaaagttgcgaaaccaaaagaatttagggttatcatactttagtaaacttggaatagaccgttcaaatatatctagatttgaacatggaaaatgtatgatgagttttgagcgtatagatttgatgttagaagaaatgcaagttccgttatctgagtacgaattgattgtaaataattttatgccgaatttccaagaattttttatattagaattggaaaaagctgaatttagccaaaatcgagataaaataaaagagttgtattctgaggtcaaagaaacggggaatcatttactgacggttaccgtgaaaacgaagcttgggaatataagtcagacagaagttaaagaaattgaagcttatctttgcaatattgaagagtggggatattttgaacttactttattttattttgtatctgattatctcaatgtcaatcaattagaattgctgctttttaattttgataaaagatgtgaaaattactgtagagtcttaaaatatagaaggagactattgcaaatagcctataaaagtgttgcgatatacgcggctaaaggagaaagaaaaaaagccgaaaatattttagaaatgactaaaaaatatcgaactgtgggagtcgatttatattcagaagtattaagacatcttgctagagctatcattatttttaattttgaaaatgcagagattggggaagaaaaaataaattatgctcttgagattttggaagaatttggaggaaagaagataaaagaattctatcagaataaaatggaaaagtatttgaaaaggtcaatttagtctcttttgagctgttgctttaaagcaacagctcaaaagagattttctttattctagagcatatactagagggtgaagataggttgtctgaagcattataacttgtcttttaaaaaattcaatcataaatataaggaggtatgatgagcaaaggagaagaagataacatggcaatcatcaaagaatttatgcgtttcaaagttcacatggaaggttctgtaaacggacacgaatttgaaattgaaggtgaaggtgaaggccgtccttatgaaggaacacaaacggcaaagctgaaagtaacaaaaggcggaccgcttccgtttgcatgggatatcctttctccgcaattcatgtacggttcaaaagcatacgtgaagcatccggctgatattcctgattatttgaagctgtcattccctgaaggcttcaaatgggagcgtgtgatgaactttgaagatggcggtgttgttactgttactcaagattcaagccttcaagacggtgaatttatttacaaagtgaagctgcgcggaacaaacttcccatctgacggacctgtcatgcaaaagaaaacaatgggctgggaagcaagctctgaacgcatgtatccagaggacggtgctttaaaaggagaaatcaaacagcgtttgaagctgaaagacggcggacactatgacgctgaagtgaaaacaacttacaaagcgaaaaagccggttcagcttccaggtgcttacaacgtaaacatcaaacttgatattacaagccacaatgaagattatacgattgttgaacaatatgaacgcgctgaaggccgtcattcaactggcggaatggatgagctttacaaataataagcatgc

SEQ ID NO: 36 - DNA, 5096 bp, Artificial Sequence
  plasmid pC-mCherry
gatctgagcgttgtataagcttttatgtctttctatatcaacttttaatagaaatataaagtaatataaatgtttttataataaattatgtgagatatatttttttgtccgtactggtatagatttgacgattaagtcttaaataagttataatctcaattgcgtaatttcttaaatacagaaataacaactacattggtagactgattaaaaagtgtacttgatgaactgttataaaccttaaaaaaataaaaataatagtttgggggatgttaaagatgtataaaaaatatggagattgttttaaaaagttgcgaaaccaaaagaatttagggttatcatactttagtaaacttggaatagaccgttcaaatatatctagatttgaacatggaaaatgtatgatgagttttgagcgtatagatttgatgttagaagaaatgcaagttccgttatctgagtacgaattgattgtaaataattttatgccgaatttccaagaattttttatattagaattggaaaaagctgaatttagccaaaatcgagataaaataaaagagttgtattctgaggtcaaagaaacggggaatcatttactgacggttaccgtgaaaacgaagcttgggaatataagtcagacagaagttaaagaaattgaagcttatctttgcaatattgaagagtggggatattttgaacttactttattttattttgtatctgattatctcaatgtcaatcaattagaattgctgctttttaattttgataaaagatgtgaaaattactgtagagtcttaaaatatagaaggagactattgcaaatagcctataaaagtgttgcgatatacgcggctaaaggagaaagaaaaaaagccgaaaatattttagaaatgactaaaaaatatcgaactgtgggagtcgatttatattcagaagtattaagacatcttgctagagctatcattatttttaattttgaaaatgcagagattggggaagaaaaaataaattatgctcttgagattttggaagaatttggaggaaagaagataaaagaattctatcagaataaaatggaaaagtatttgaaaaggtcaatttagtctcttttgagctgttgctttaaagcaacagctcaaaagagattttctttattctagagcatatactagagggtgaagataggttgtctgaagcattataacttgtcttttaaaaaattcaatcataaatataaggaggtatgatgagcaaaggagaagaagataacatggcaatcatcaaagaatttatgcgtttcaaagttcacatggaaggttctgtaaacggacacgaatttgaaattgaaggtgaaggtgaaggccgtccttatgaaggaacacaaacggcaaagctgaaagtaacaaaaggcggaccgcttccgtttgcatgggatatcctttctccgcaattcatgtacggttcaaaagcatacgtgaagcatccggctgatattcctgattatttgaagctgtcattccctgaaggcttcaaatgggagcgtgtgatgaactttgaagatggcggtgttgttactgttactcaagattcaagccttcaagacggtgaatttatttacaaagtgaagctgcgcggaacaaacttcccatctgacggacctgtcatgcaaaagaaaacaatgggctgggaagcaagctctgaacgcatgtatccagaggacggtgctttaaaaggagaaatcaaacagcgtttgaagctgaaagacggcggacactatgacgctgaagtgaaaacaacttacaaagcgaaaaagccggttcagcttccaggtgcttacaacgtaaacatcaaacttgatattacaagccacaatgaagattatacgattgttgaacaatatgaacgcgctgaaggccgtcattcaactggcggaatggatgagctttacaaataataagcatgcggtaccactagttctagagagctcaagctttctttgaaccaaaattagaaaaccaaggcttgaaacgttcaattgaaatggcaattaaacaaattacagcacgtgttgctttgattgatagccaaaaagcagcagttgataaagcaattactgatattgctgaaaaattgtaatttataaataaaaatcaccttttagaggtggtttttttatttataaattattcgtttgatttcgctttcgatagaacaatcaaatcgtttctgagacgttttagcgtttatttcgtttagttatcggcataatcgttaaaacaggcgttatcgtagcgtaaaagcccttgagcgtagcgtggctttgcagcgaagatgttgtctgttagattatgaaagccgatgactgaatgaaataataagcgcagcgtccttctatttcggttggaggaggctcaagggagtttgagggaatgaaattccctcatgggtttgattttaaaaattgcttgcaattttgccgagcggtagcgctggaaaatttttgaaaaaaatttggaatttggaaaaaaatggggggaaaggaagcgaattttgcttccgtactacgaccccccattaagtgccgagtgccaatttttgtgccaaaaacgctctatcccaactggctcaagggtttgaggggtttttcaatcgccaacgaatcgccaacgttttcgccaacgttttttataaatctatatttaagtagctttatttttgtttttatgattacaaagtgatacactaattttataaaattatttgattggagttttttaaatggtgatttcagaatcgaaaaaaagagttatgatttctctgacaaaagagcaagataaaaaattaacagatatggcgaaacaaaaagatttttcaaaatctgcggttgcggcgttagctatagaagaatatgcaagaaaggaatcagaacaaaaaaaataagcgaaagctcgcgtttttagaaggatacgagttttcgctacttgtttttgataaggtaattatatcatggctattaaaaatactaaagctagaaattttggatttttattatatcctgactcaattcctaatgattggaaagaaaaattagagagtttgggcgtatctatggctgtcagtcctttacacgatatggacgaaaaaaaagataaagatacatggaatagtagtgatgttatacgaaatggaaagcactataaaaaaccacactatcacgttatatatattgcacgaaatcctgtaacaatagaaagcgttaggaacaagattaagcgaaaattggggaatagttcagttgctcatgttgagatacttgattatatcaaaggttcatatgaatatttgactcatgaatcaaaggacgctattgctaagaataaacatatatacgacaaaaaagatattttgaacattaatgattttgatattgaccgctatataacacttgatgaaagccaaaaaagagaattgaagaatttacttttagatatagtggatgactataatttggtaaatacaaaagatttaatggcttttattcgccttaggggagcggagtttggaattttaaatacgaatgatgtaaaagatattgtttcaacaaactctagcgcctttagattatggtttgagggcaattatcagtgtggatatagagcaagttatgcaaaggttcttgatgctgaaacgggggaaataaaatgacaaacaaagaaaaagagttatttgctgaaaatgaggaattaaaaaaagaaattaaggacttaaaagagcgtattgaaagatacagagaaatggaagttgaattaagtacaacaatagatttattgagaggagggattattgaataaataaaagcccccctgacgaaagtcgacatggtcgatgtctagatgcttaaactagagaaaggtttaaaagatgaaaacttcaccacatcgtaatacttcagctattgttgatttaaaagcgattagaaataatattgaaaaatttaaaaagcatattaaccctaatgcagagatttggccagcagtgaaagcagatgcttatggtcatggctcgattgaggtttctaaagcggtgagcgatttggtaggtggtttttgtgtatcaaacctagatgaggcaattgaattacgaaatcatctggtgactaaaccgattttagttttatccggaattgttccagaagatgttgatattgcagctgcccttaatattagtcttactgccccgagtttagaatggttgaaattggttgttcaagaagaagcagaactttcagatttaaaaattcatattggtgtagattctggtatgggtcggattggtattcgtgatgttgaagaagctaatcagatgattgaacttgctgataaatatgcgattaattttgaaggaattttcactcattttgcgactgcggatatggctgatgaaacaaaatttaaaaatcaacaggcaagatttaacaaaattatggccggattatcacgtcaaccaaaatttatacactcaactaatacggccgctgctttatggcataaggaacaagttcaagctattgaacgtttagggatttcaatgtatggcttgaatccaagtggtaaaactttggaacttccttttgaaattgaacccgctctctctttagtttctgaattgactcatataaaaaaaatagctgcaggtgaaacggttggttatggtgcaacttatgagacgagtgaagaaacttggattggaactgttccaattggttacgctgacgggtggacccgtcaaatgcaaggtttcaaagtgcttgttgatggaaagttttgtgagattgttggtcgagtttgtatggatcaaatgatgataaaacttgataagtcttaccctttgggaacgaaggtcactttgattggtcgagataaggctaatgaaatcacgacaacagacgttgctgattggcgtggaacgattaattatgaagtgctttgcttactttctgatagaatcaaaagaatctataaataaaattaaaaaaactgtatttttacagtttttttgttttctgttaaaagcagatgataacctcacta